European Patent Specification EP 3 800 271 B1, published October 30, 2024. Title: Improving the Level of Hydration in a Cat. Applicant: Hill's Pet Nutrition, Inc. The sequence listing filed with the application follows.

SEQUENCE LISTING (3 sequences)

SEQ ID NO: 1 - DNA, 201 bp, Felis catus
attttagaaatctaccaccgtatggaggcaagtgtagagggattcttagccgagggtagaagaactattaggaaatgatagcaatagcctgttcaggtggytctcagttaaggcagtggcattaggaatgaagcaatggggggataaacagaaaatatttagaaagtaaatatagtagggaatggctatgaagaagtctgt

SEQ ID NO: 2 - DNA, 201 bp, Felis catus
ataaattaaacttctgtccaagatgatgagtgcatgcaagaaagcaccactcacaaaaaaatgggatagggacaccataatggagtgaggacctttactcrggctgggaaatcttcccaccctccagtctggaagttttattttggtgaaccctctaaagatacaaggtacaggaacaccagcttccagcaccataaaaat

SEQ ID NO: 3 - DNA, 201 bp, Felis catus
cagtggagagtcgaagtttgtgggaatggggagatgagatgaggacactccttgtcttcaggcacatcattagggggagaaggttacccatctgttttcarccattatctcttgaactgccgctttgtcccttgaacgtggttgggctgtaatgagggatagtaaccaagagaatgaaaacagtacttactgcctattgta